European Patent Application EP 4 656 203 A1, published December 3, 2025. Title: COMPOSITIONS AND METHODS FOR OPTIMIZED IGG PRODUCTION. Applicant: ABBRATECH INC. Application EP. The sequence listing filed with the application follows.

SEQUENCE LISTING (19 sequences)

SEQ ID NO: 1 - protein, 14 aa, Synthetic construct
EQELLELDKWASLW

SEQ ID NO: 2 - protein, 14 aa, Synthetic construct
  MOD_RES 8: note = An amino acid
EQELLELXKWASLW

SEQ ID NO: 3 - protein, 7 aa, Synthetic construct
GGGSGSS

SEQ ID NO: 4 - protein, 9 aa, Synthetic construct
YPYDVPDYA

SEQ ID NO: 5 - protein, 5 aa, Synthetic construct
LPETG

SEQ ID NO: 6 - DNA, 15 bp, Synthetic construct
  source 1..15: mol_type = other DNA
ttaccggaaactggt

SEQ ID NO: 7 - protein, 5 aa, Synthetic construct
GGGGS

SEQ ID NO: 8 - DNA, 15 bp, Synthetic construct
  source 1..15: mol_type = other DNA
ggtggcggtggctcg

SEQ ID NO: 9 - protein, 9 aa, Synthetic construct
YPYDVPDYA

SEQ ID NO: 10 - protein, 33 aa, Synthetic construct
  MOD_RES 17: note = Phosphoserine
GGGSGSSERRPHFPQFXYSASGTAYPYDVPDYA

SEQ ID NO: 11 - protein, 33 aa, Synthetic construct
GGGSGSSERRPHFPQFSYSASGTAYPYDVPDYA

SEQ ID NO: 12 - protein, 24 aa, Synthetic construct
MLMGGRGSGSEQELLELDKWASLW

SEQ ID NO: 13 - protein, 24 aa, Synthetic construct
MLMGGRGSGSEQELLELEKWASLW

SEQ ID NO: 14 - DNA, 30 bp, Synthetic construct
  source 1..30: mol_type = other DNA
ggtggcggtggctcgttaccggaaactggt

SEQ ID NO: 15 - protein, 6 aa, Synthetic construct
ELDKWA

SEQ ID NO: 16 - protein, 4 aa, Synthetic construct
GSGS

SEQ ID NO: 17 - protein, 5 aa, Synthetic construct
GSGSG

SEQ ID NO: 18 - protein, 6 aa, Synthetic construct
GSGSGS

SEQ ID NO: 19 - protein, 34 aa, Synthetic construct
QNQQEKNEQELLELDKWASLWNWFNITNWLWYIK